European Patent Application EP 4 239 334 A1, published September 6, 2023. Title: SEPARATION-OF-FUNCTION IKBα MUTANTS. Applicant: Consorcio Centro de Investigación Biomédica en Red (CIBER). The sequence listing filed with the application follows.

SEQUENCE LISTING (4 sequences)

SEQ ID NO: 1 - protein, 317 aa, Artificial sequence
  Artificial sequence
MFQAAERPQEWAMEGPRDGLKKERLLDDRHDSGLDSMKDEEYEQMVKELQEIRLEPQEVPRGSEPWKQQLTEDGDSFLHLAIIAAAKALTMEVIRQVKGDLAFLNFQNNLQQTPLHLAVITNQPEIAEALLGAGCDPELRDFRGNTPLHLACEQGCLASVGVLTQSCTTPHLHSILKATNYNGHTCLHLASIHGYLGIVELLVSLGADVNAQEPCNGRTALHLAVDLQNPDLVSLLLKCGADVNRVTYQGYSPYQLTWGRPSTRIQQQLGQLTLENLQMLPESEDEESYDTESEFTEFTEDELPYDDCVFGGQRLTL

SEQ ID NO: 2 - protein, 317 aa, Artificial sequence
  Artificial sequence
MFQAAERPQEWAMEGPRDGLKKERLLDDRHDSGLDSMKDEEYEQMVKELQEIRLEPQEVPRGSEPWKQQLTEDGASFLHLAIIHEEKALTMEVIRQVKGDLAFLNFQNNLQQTPLHLAVITNQPEIAEALLGAGCDPELRDFRGNTPLHLACEQGCLASVGVLTQSCTTPHLHSILKATNYNGHTCLHLASIHGYLGIVELLVSLGADVNAQEPCNGRTALHLAVDLQNPDLVSLLLKCGADVNRVTYQGYSPYQLTWGRPSTRIQQQLGQLTLENLQMLPESEDEESYDTESEFTEFTEDELPYDDCVFGGQRLTL

SEQ ID NO: 3 - protein, 317 aa, Artificial sequence
  Artificial sequence
MFQAAERPQEWAMEGPRDGLKKERLLDDRHDSGLDSMKDEEYEQMVKELQEIRLEPQEVPRGSEPWKQQLTEDGDSFLHLAIIHEEKALTMEVIRQVKGDLAFLNFQANLQQTPLHLAVITNQPEIAEALLGAGCDPELRDFRGNTPLHLACEQGCLASVGVLTQSCTTPHLHSILKATNYNGHTCLHLASIHGYLGIVELLVSLGADVNAQEPCNGRTALHLAVDLQNPDLVSLLLKCGADVNRVTYQGYSPYQLTWGRPSTRIQQQLGQLTLENLQMLPESEDEESYDTESEFTEFTEDELPYDDCVFGGQRLTL

SEQ ID NO: 4 - protein, 317 aa, Artificial sequence
  Artificial sequence
MFQAAERPQEWAMEGPRDGLKKERLLDDRHDSGLDSMKDEEYEQMVKELQEIRLEPQEVPRGSEPWKQQLTEDGDSFLHLAIIHEEKALTMEVIRQVKGDLAFLNFQNNLQQTPLHLAVITNQPEIAEALLGAGCDPELRDFRGNTPLHLACEQGCLASVGVLTQSCTTPHLHSILKATNYNGHTCLHLASIHGYLGIVELLVSLGADVNAQEPCNGRTALHLAVDLQNPDLVSLLLKCGADVNRVTYQGYSPYQLTWGRPSTRIQQQLGQLTLENLQMLPESEDEESYDTESEFTEFTEDELPYDDCVFGGQRLTL